European Patent Application EP 4 454 657 A1, published October 30, 2024. Title: Hepatic targeting agent and use thereof. Applicant: HANMI PHARM. CO., LTD. The sequence listing filed with the application follows.

SEQUENCE LISTING (71 sequences)

SEQ ID NO: 1 - protein, 29 aa, Homo sapiens
HSQGTFTSDYSKYLDSRRAQDFVQWLMNT

SEQ ID NO: 2 - protein, 29 aa, synthetic construct
  REGION 1..29: note = glucagon derivative
HSQGTFTSDYSKYLDCDRAQDFVQWLMNT

SEQ ID NO: 3 - protein, 29 aa, synthetic construct
  REGION 1..29: note = glucagon derivative
HSQGTFTSDYSKYLDCERAQDFVQWLMNT

SEQ ID NO: 4 - protein, 29 aa, synthetic construct
  REGION 1..29: note = glucagon derivative
HSQGTFTSDYSKYLDSCDAQDFVQWLMNT

SEQ ID NO: 5 - protein, 29 aa, synthetic construct
  REGION 1..29: note = glucagon derivative
HSQGTFTSDYSKYLDSCEAQDFVQWLMNT

SEQ ID NO: 6 - protein, 29 aa, synthetic construct
  REGION 1..29: note = glucagon derivative
HSQGTFTSDYSKYLDSCEADDFVQWLMNT

SEQ ID NO: 7 - protein, 29 aa, synthetic construct
  REGION 1..29: note = glucagon derivative
YSQGTFTSDYSKYLDSCEADDFVQWLMNT

SEQ ID NO: 8 - protein, 29 aa, synthetic construct
  REGION 1..29: note = glucagon derivative
  SITE 2: note = X is aminoisobutyric acid (Aib)
YXQGTFTSDYSKYLDSCDAQDFVQWLINT

SEQ ID NO: 9 - protein, 29 aa, synthetic construct
  REGION 1..29: note = glucagon derivative
  SITE 2: note = X is aminoisobutyric acid (Aib)
YXQGTFTSDYSKYLDSCDAQDFVVWLINT

SEQ ID NO: 10 - protein, 29 aa, synthetic construct
  REGION 1..29: note = glucagon derivative
  SITE 2: note = X is aminoisobutyric acid (Aib)
YXQGTFTSDYSKYLDSCDADDFVVWLINT

SEQ ID NO: 11 - protein, 29 aa, synthetic construct
  REGION 1..29: note = glucagon derivative
  SITE 2: note = X is aminoisobutyric acid (Aib)
YXQGTFTSDYSKYLDEKCAKEFVQWLMNT

SEQ ID NO: 12 - protein, 30 aa, synthetic construct
  REGION 1..30: note = glucagon derivative
  SITE 2: note = X is aminoisobutyric acid (Aib)
  SITE 16..20: note = amino acids at positions 16 and 20 together form a ring
YXQGTFTSDYSKYLDEKRAKEFVQWLMNTC

SEQ ID NO: 13 - protein, 29 aa, synthetic construct
  REGION 1..29: note = glucagon derivative
  SITE 2: note = X is aminoisobutyric acid (Aib)
YXQGTFTSDYSCYLDSRRAQDFVQWLMNT

SEQ ID NO: 14 - protein, 29 aa, synthetic construct
  REGION 1..29: note = glucagon derivative
  SITE 2: note = X is aminoisobutyric acid (Aib)
YXQGTFTSDYSKYLDCKRAKEFVQWLMNT

SEQ ID NO: 15 - protein, 29 aa, synthetic construct
  REGION 1..29: note = glucagon derivative
  SITE 2: note = X is aminoisobutyric acid (Aib)
YXQGTFTSDYSKYLCEKRAQDFVVWLMNT

SEQ ID NO: 16 - protein, 29 aa, synthetic construct
  REGION 1..29: note = glucagon derivative
  SITE 2: note = X is aminoisobutyric acid (Aib)
YXQGTFTSDYSKYLDCRRAQVFVQWLMRT

SEQ ID NO: 17 - protein, 29 aa, synthetic construct
  REGION 1..29: note = glucagon derivative
  SITE 2: note = X is aminoisobutyric acid (Aib)
YXQGTFTSDYSKYLDCVRAQDFVQWLMRT

SEQ ID NO: 18 - protein, 29 aa, synthetic construct
  REGION 1..29: note = glucagon derivative
  SITE 2: note = X is aminoisobutyric acid (Aib)
YXQGTFTSDYSKYLDSRRACDFRLWLMNT

SEQ ID NO: 19 - protein, 29 aa, synthetic construct
  REGION 1..29: note = glucagon derivative
  SITE 2: note = X is aminoisobutyric acid (Aib)
  SITE 16..20: note = amino acids at positions 16 and 20 together form a ring
YXQGTFTSDYSKYLCEKRAKEFVQWLMNT

SEQ ID NO: 20 - protein, 29 aa, synthetic construct
  REGION 1..29: note = glucagon derivative
  SITE 2: note = X is aminoisobutyric acid (Aib)
  SITE 16..20: note = amino acids at positions 16 and 20 together form a ring
YXQGTFTSDYSKYLDECRAKEFVQWLMNT

SEQ ID NO: 21 - protein, 29 aa, synthetic construct
  REGION 1..29: note = glucagon derivative
  SITE 2: note = X is aminoisobutyric acid (Aib)
  SITE 16..20: note = amino acids at positions 16 and 20 together form a ring
YXQGTFTSDYSKYLDEKCAKEFVQWLMNT

SEQ ID NO: 22 - protein, 29 aa, synthetic construct
  REGION 1..29: note = glucagon derivative
  SITE 2: note = X is aminoisobutyric acid (Aib)
  SITE 16..20: note = amino acids at positions 16 and 20 together form a ring
YXQGTFTSDYSKYLDEKRCKEFVQWLMNT

SEQ ID NO: 23 - protein, 29 aa, synthetic construct
  REGION 1..29: note = glucagon derivative
  SITE 2: note = X is aminoisobutyric acid (Aib)
  REGION 16..20: note = amino acids at positions 16 and 20 together form a ring
YXQGTFTSDYSKYCDEKRAKEFVQWLMNT

SEQ ID NO: 24 - protein, 29 aa, synthetic construct
  REGION 1..29: note = glucagon derivative
  SITE 2: note = X is aminoisobutyric acid (Aib)
  SITE 16..20: note = amino acids at positions 16 and 20 together form a ring
YXQGTFTSDYSKCLDEKRAKEFVQWLMNT

SEQ ID NO: 25 - protein, 29 aa, synthetic construct
  REGION 1..29: note = glucagon derivative
  SITE 2: note = X is aminoisobutyric acid (Aib)
  SITE 16..20: note = amino acids at positions 16 and 20 together form a ring
YXQGTFTSDYSKYLDEKRAKCFVQWLMNT

SEQ ID NO: 26 - protein, 29 aa, synthetic construct
  REGION 1..29: note = glucagon derivative
  SITE 2: note = X is aminoisobutyric acid (Aib)
  SITE 16..20: note = amino acids at positions 16 and 20 together form a ring
WXQGTFTSDYSKYLDECRAKDFVQWLMNT

SEQ ID NO: 27 - protein, 29 aa, synthetic construct
  REGION 1..29: note = glucagon derivative
  SITE 2: note = X is aminoisobutyric acid (Aib)
  REGION 16..20: note = amino acids at positions 16 and 20 together form a ring
YXQGTFVSDYSKYLDECRAKDFVQWLMNT

SEQ ID NO: 28 - protein, 29 aa, synthetic construct
  REGION 1..29: note = glucagon derivative
  SITE 2: note = X is aminoisobutyric acid (Aib)
  SITE 16..20: note = amino acids at positions 16 and 20 together form a ring
WXQGTFVSDYSKYLDECRAKDFVQWLMNT

SEQ ID NO: 29 - protein, 29 aa, synthetic construct
  REGION 1..29: note = glucagon derivative
  SITE 2: note = X is aminoisobutyric acid (Aib)
  SITE 16..20: note = amino acids at positions 16 and 20 together form a ring
YXQGTFTSDYSKCLDERRAKDFVQWLMNT

SEQ ID NO: 30 - protein, 29 aa, synthetic construct
  REGION 1..29: note = glucagon derivative
  SITE 2: note = X is aminoisobutyric acid (Aib)
  SITE 16..20: note = amino acids at positions 16 and 20 together form a ring
WXQGTFTSDYSKCLDERRAKDFVQWLMNT

SEQ ID NO: 31 - protein, 29 aa, synthetic construct
  REGION 1..29: note = glucagon derivative
  SITE 2: note = X is aminoisobutyric acid (Aib)
  SITE 17..21: note = amino acids at positions 17 and 21 together form a ring
YXQGTFTSDYSKYLDCKRAKEFVQWLMNT

SEQ ID NO: 32 - protein, 28 aa, synthetic construct
  REGION 1..28: note = glucagon derivative
  SITE 15..19: note = amino acids at positions 15 and 19 together form a ring
SQGTFTSDYSKYLDECRAKEFVQWLMNT

SEQ ID NO: 33 - protein, 29 aa, synthetic construct
  REGION 1..29: note = glucagon derivative
  SITE 2: note = X is aminoisobutyric acid (Aib)
YXQGTFTSDYSKYLDSRRAQDFVQWLMNT

SEQ ID NO: 34 - protein, 29 aa, synthetic construct
  REGION 1..29: note = glucagon derivative
  SITE 2: note = X is aminoisobutyric acid (Aib)
  SITE 16..20: note = amino acids at positions 16 and 20 together form a ring
WXQGTFTSDYSKYCDERRAKEFVQWLMNT

SEQ ID NO: 35 - protein, 29 aa, synthetic construct
  REGION 1..29: note = glucagon derivative
  SITE 2: note = X is aminoisobutyric acid (Aib)
  REGION 16..20: note = amino acids at positions 16 and 20 together form a ring
YXQGTFTSDYSKYCDERRAKEFVQWLMNT

SEQ ID NO: 36 - protein, 29 aa, synthetic construct
  REGION 1..29: note = glucagon derivative
  SITE 2: note = X is aminoisobutyric acid (Aib)
  SITE 16..20: note = amino acids at positions 16 and 20 together form a ring
YXQGTFTSDCSKYLDERRAKEFVQWLMNT

SEQ ID NO: 37 - protein, 30 aa, synthetic construct
  REGION 1..30: note = glucagon derivative
  SITE 2: note = X is aminoisobutyric acid (Aib)
  SITE 16..20: note = amino acids at positions 16 and 20 together form a ring
YXQGTFTSDYSKYLDERRAKEFVQWLMNTC

SEQ ID NO: 38 - protein, 29 aa, synthetic construct
  REGION 1..29: note = glucagon derivative
  SITE 2: note = X is aminoisobutyric acid (Aib)
  SITE 16..20: note = amino acids at positions 16 and 20 together form a ring
YXQGTFCSDYSKYLDERRAKEFVQWLMNT

SEQ ID NO: 39 - protein, 29 aa, synthetic construct
  REGION 1..29: note = glucagon derivative
  SITE 2: note = X is aminoisobutyric acid (Aib)
  SITE 16..20: note = amino acids at positions 16 and 20 together form a ring
YXQGTFVSDCSKYLDERRAKDFVQWLMNT

SEQ ID NO: 40 - protein, 30 aa, synthetic construct
  REGION 1..30: note = glucagon derivative
  SITE 2: note = X is aminoisobutyric acid (Aib)
  REGION 16..20: note = amino acids at positions 16 and 20 together form a ring
YXQGTFVSDYSKYLDERRAKDFVQWLMNTC

SEQ ID NO: 41 - protein, 29 aa, synthetic construct
  REGION 1..29: note = glucagon derivative
  SITE 2: note = X is aminoisobutyric acid (Aib)
  SITE 16..20: note = amino acids at positions 16 and 20 together form a ring
YXQGTFCSDYSKYLDERRAKDFVQWLMNT

SEQ ID NO: 42 - protein, 29 aa, synthetic construct
  REGION 1..29: note = glucagon derivative
  SITE 2: note = X is aminoisobutyric acid (Aib)
YXQGTFCSDYSKYLDSRRAQDFVQWLMNT

SEQ ID NO: 43 - protein, 29 aa, synthetic construct
  REGION 1..29: note = glucagon derivative
  SITE 2: note = X is aminoisobutyric acid (Aib)
YXQGTFTSDCSKYLDSRRAQDFVQWLMNT

SEQ ID NO: 44 - protein, 30 aa, synthetic construct
  REGION 1..30: note = glucagon derivative
  SITE 2: note = X is aminoisobutyric acid (Aib)
YXQGTFTSDYSKYLDSRRAQDFVQWLMNTC

SEQ ID NO: 45 - protein, 29 aa, synthetic construct
  REGION 1..29: note = Glucagon analog
  SITE 2: note = X is aminoisobutyric acid (Aib)
YXQGTFTSDYSCYLDEKRAKEFVQWLMNT

SEQ ID NO: 46 - protein, 30 aa, synthetic construct
  REGION 1..30: note = glucagon derivative
  SITE 1: note = X is histidine, desamino-histidyl, N-dimethyl-histidyl, beta-hydroxy imidazopropionyl, 4-imidazoacetyl, beta-carboxy imidazopropionyl, tryptophan, or tyrosine, or is absent
  SITE 2: note = X is alpha-methyl-glutamic acid, aminoisobutyric acid (Aib), D-alanine, glycine, Sar (N-methylglycine), serine, or D-serine
  SITE 7: note = X is threonine, valine, or cysteine
  SITE 10: note = X is tyrosine or cysteine
  SITE 12: note = X is lysine or cysteine
  SITE 13: note = X is tyrosine or cysteine
  SITE 14: note = X is leucine or cysteine
  SITE 15: note = X is aspartic acid, glutamic acid, or cysteine
  SITE 16: note = X is glutamic acid, aspartic acid, serine, alpha-methyl-glutamic acid, or cysteine, or is absent;
  SITE 17: note = X is aspartic acid, glutamine, glutamic acid, lysine, arginine, serine, cysteine, or valine, or is absent
  SITE 18: note = X is alanine, aspartic acid, glutamine, glutamic acid, arginine, valine, or cysteine, or is absent
  SITE 19: note = X is alanine, arginine, serine, valine, or cysteine, or is absent
  SITE 20: note = X is lysine, histidine, glutamic acid, glutamine, aspartic acid, arginine, alpha-methyl-glutamic acid, or cysteine, or is absent
  SITE 21: note = X is aspartic acid, glutamic acid, leucine, valine, or cysteine, or is absent
  SITE 23: note = X is isoleucine, valine, or arginine, or is absent
  SITE 24: note = X is valine, arginine, alanine, cysteine, glutamic acid, lysine, glutamine, alpha-methyl-glutamic acid, or leucine, or is absent;
  SITE 27: note = X is isoleucine, valine, alanine, lysine, methionine, glutamine, or arginine, or is absent
  SITE 28: note = X is glutamine, lysine, asparagine, or arginine, or is absent
  SITE 29: note = X is lysine, alanine, glycine, or threonine, or is absent
  SITE 30: note = X is cysteine, or is absent
XXQGTFXSDXSXXXXXXXXXXFXXWLXXXX

SEQ ID NO: 47 - protein, 30 aa, synthetic construct
  REGION 1..30: note = glucagon derivative
  SITE 2: note = X is aminoisobutyric acid (Aib)
  SITE 7: note = X is threonine, valine, or cysteine
  SITE 10: note = X is tyrosine or cysteine
  SITE 12: note = X is lysine or cysteine
  SITE 15: note = X is aspartic acid or cysteine
  SITE 16: note = X is glutamic acid or serine
  SITE 17: note = X is lysine or arginine
  SITE 20: note = X is glutamine or lysine
  SITE 21: note = X is aspartic acid or glutamic acid
  SITE 24: note = X is valine or glutamine
  SITE 30: note = X is cysteine or is absent
YXQGTFXSDXSXYLXXXRAXXFVXWLMNTX

SEQ ID NO: 48 - DNA, 34 bp, synthetic construct
  misc_feature 1..34: note = Forward primer
  source 1..34: mol_type = other DNA
cagcgacaccgaccgtccccccgtacttaaggcc

SEQ ID NO: 49 - DNA, 32 bp, synthetic construct
  misc_feature 1..32: note = Reverse primer
  source 1..32: mol_type = other DNA
ctaaccgactctcggggaagactgagctcgcc

SEQ ID NO: 50 - protein, 12 aa, Homo sapiens
ESKYGPPCPSCP

SEQ ID NO: 51 - protein, 11 aa, synthetic construct
  REGION 1..11: note = Variant of hinge region
ESKYGPPPSCP

SEQ ID NO: 52 - protein, 11 aa, synthetic construct
  REGION 1..11: note = Variant of hinge region
ESKYGPPCPSP

SEQ ID NO: 53 - protein, 10 aa, synthetic construct
  REGION 1..10: note = Variant of hinge region
ESKYGPPCPS

SEQ ID NO: 54 - protein, 10 aa, synthetic construct
  REGION 1..10: note = Variant of hinge region
ESKYGPPCPP

SEQ ID NO: 55 - protein, 8 aa, synthetic construct
  REGION 1..8: note = Variant of hinge region
KYGPPCPS

SEQ ID NO: 56 - protein, 8 aa, synthetic construct
  REGION 1..8: note = Variant of hinge region
ESKYGPPC

SEQ ID NO: 57 - protein, 7 aa, synthetic construct
  REGION 1..7: note = Variant of hinge region
EKYGPPC

SEQ ID NO: 58 - protein, 6 aa, synthetic construct
  REGION 1..6: note = Variant of hinge region
ESPSCP

SEQ ID NO: 59 - protein, 5 aa, synthetic construct
  REGION 1..5: note = Variant of hinge region
EPSCP

SEQ ID NO: 60 - protein, 4 aa, synthetic construct
  REGION 1..4: note = Variant of hinge region
PSCP

SEQ ID NO: 61 - protein, 10 aa, synthetic construct
  REGION 1..10: note = Variant of hinge region
ESKYGPPSCP

SEQ ID NO: 62 - protein, 9 aa, synthetic construct
  REGION 1..9: note = Variant of hinge region
KYGPPPSCP

SEQ ID NO: 63 - protein, 9 aa, synthetic construct
  REGION 1..9: note = Variant of hinge region
ESKYGPSCP

SEQ ID NO: 64 - protein, 8 aa, synthetic construct
  REGION 1..8: note = Variant of hinge region
ESKYGPPC

SEQ ID NO: 65 - protein, 7 aa, synthetic construct
  REGION 1..7: note = Variant of hinge region
KYGPPCP

SEQ ID NO: 66 - protein, 7 aa, synthetic construct
  REGION 1..7: note = Variant of hinge region
ESKPSCP

SEQ ID NO: 67 - protein, 6 aa, synthetic construct
  REGION 1..6: note = Variant of hinge region
ESPSCP

SEQ ID NO: 68 - protein, 4 aa, synthetic construct
  REGION 1..4: note = Variant of hinge region
EPSC

SEQ ID NO: 69 - skipped

SEQ ID NO: 70 - protein, 221 aa, Homo sapiens
PSCPAPEFLGGPSVFLFPPKPKDTLMISRTPEVTCVVVDVSQEDPEVQFNWYVDGVEVHNAKTKPREEQFNSTYRVVSVLTVLHQDWLNGKEYKCKVSNKGLPSSIEKTISKAKGQPREPQVYTLPPSQEEMTKNQVSLTCLVKGFYPSDIAVEWESNGQPENNYKTTPPVLDSDGSFFLYSRLTVDKSRWQEGNVFSCSVMHEALHNHYTQKSLSLSLGK

SEQ ID NO: 71 - protein, 442 aa, Homo sapiens
  REGION 1..442: note = Amino acids at position 1 to 442 form Human Immunoglobulin G4 Fc Fragment (homodimer)
  REGION 1..221: note = Amino acids at position 1 to 221 form one monomer
  REGION 222..442: note = Amino acids at position 222 to 442 form one monomer
  DISULFID 3..224: note = Amino acids at position 3 and position 224 form an inter-disulfide bond
  DISULFID 35..95: note = Amino acids at position 35 and position 95 form an intra-chain disulfide bond
  DISULFID 141..199: note = Amino acids at position 141 and position 199 form an intra-chain disulfide bond
  DISULFID 256..316: note = Amino acids at position 256 and position 316 form an intra-chain disulfide bond
  DISULFID 362..420: note = Amino acids at position 362 and position 420 form an intra-chain disulfide bond
PSCPAPEFLGGPSVFLFPPKPKDTLMISRTPEVTCVVVDVSQEDPEVQFNWYVDGVEVHNAKTKPREEQFNSTYRVVSVLTVLHQDWLNGKEYKCKVSNKGLPSSIEKTISKAKGQPREPQVYTLPPSQEEMTKNQVSLTCLVKGFYPSDIAVEWESNGQPENNYKTTPPVLDSDGSFFLYSRLTVDKSRWQEGNVFSCSVMHEALHNHYTQKSLSLSLGKPSCPAPEFLGGPSVFLFPPKPKDTLMISRTPEVTCVVVDVSQEDPEVQFNWYVDGVEVHNAKTKPREEQFNSTYRVVSVLTVLHQDWLNGKEYKCKVSNKGLPSSIEKTISKAKGQPREPQVYTLPPSQEEMTKNQVSLTCLVKGFYPSDIAVEWESNGQPENNYKTTPPVLDSDGSFFLYSRLTVDKSRWQEGNVFSCSVMHEALHNHYTQKSLSLSLGK